European Patent Application EP 4 317 461 A1, published February 7, 2024. Title: Microorganisms producing cyclic lipopeptide compounds and method for producing cyclic lipopeptide compounds. Applicant: KANEKA CORPORATION. The sequence listing filed with the application follows.

SEQUENCE LISTING (9 sequences)

SEQ ID NO: 1 - DNA, 1473 bp, Bacillus subtilis
atgagtcaaacattattcattgacggagaatggatcagtgccgaaaaagaacagatccgcagtattatcaacccatttaatcaagaagaaattgcaactgtaagcgagggagggcgagaggacgccatcaaagcaatcgcagccgcacgtagagcatttgacaaaggagaatggtcatcgctatccgggcttgaacgcggaaaaattgttctgaaaattgcggaattaatcagacgcgatcttgaggagctggctgagcttgaatctcttgatacaggaaaaacactcgaagaaagcaaggccgatatggacgatatcgccaatgtttttcaatattacgccggcttggcagacaaagatggcggagagatcatttcatctccgattcctgattcagaaagcaaaattattagggagccaatcggggtttgcggccagatcactccatggaattatccgctccttcaagcgagctggaaaatcgcccctgcactggccgcaggaaacacaatcgtcatgaagccgagtgagattacgccgctgacgacaatcaaagtctttaagctgatggaagaagccggtgttccaaaaggtgtcgcaaatcttgttcttggaccgggagccacagtgggcgacgagcttgccgtaaacaaagacgtcgatttgatttcatttacgggcggaattgaaacaggcaaaaaaatcatgcgggcggcaagcggaaacgtcaaaaaaatcgcccttgaacttggcgggaaaaacccaaatattgttttcaaggacgcggatttagaagttgcggttgatcaggccttaaacgctgtatttttccacgccggccaagtatgctctgcaggttcccgcttgcttgttgaggatgccattcatgatcaatttttggcggagctggtcaaacgggcaaaacgcataaaactcggaaacggttttcatgctgagacagaaagcggtccgcttatttcggcggagcacagggcaaaggtagaaaaatatgtagagatcggaatagaggaaggcgcgaagctggagacaggaggcaaacgcccggaagatcctgagcttcaaaacggctttttctatgaacctactattttctcaaactgtaattctgacatgagaatcgttcaggaagaggttttcggtcctgtattgacagtcgaaaccttcagctctgaagaagaggtaatcgagcttgcgaatgataccatctatggcttggctggagcggtatggtcaaaagacattgaaaagtgcgaacgggtagcagcccgcttgagaatgggaaccgtttggatcaacgattttcatccgtactttgcacaagcgccatggggcggatataagcaatccgggttcggacgcgagcttggaaaaataggccttgaagaatacacagaagtcaaacatgtataccgcaatacaaaaccggcagcggttaactggtttaattcataa

SEQ ID NO: 2 - protein, 490 aa, Bacillus subtilis
MSQTLFIDGEWISAEKEQIRSIINPFNQEEIATVSEGGREDAIKAIAAARRAFDKGEWSSLSGLERGKIVLKIAELIRRDLEELAELESLDTGKTLEESKADMDDIANVFQYYAGLADKDGGEIISSPIPDSESKIIREPIGVCGQITPWNYPLLQASWKIAPALAAGNTIVMKPSEITPLTTIKVFKLMEEAGVPKGVANLVLGPGATVGDELAVNKDVDLISFTGGIETGKKIMRAASGNVKKIALELGGKNPNIVFKDADLEVAVDQALNAVFFHAGQVCSAGSRLLVEDAIHDQFLAELVKRAKRIKLGNGFHAETESGPLISAEHRAKVEKYVEIGIEEGAKLETGGKRPEDPELQNGFFYEPTIFSNCNSDMRIVQEEVFGPVLTVETFSSEEEVIELANDTIYGLAGAVWSKDIEKCERVAARLRMGTVWINDFHPYFAQAPWGGYKQSGFGRELGKIGLEEYTEVKHVYRNTKPAAVNWFNS

SEQ ID NO: 3 - DNA, 1209 bp, Bacillus subtilis
atgacattaaatatgaaggtagaaagcatgcagaaattccacacatttgaaattccgactgtgattaagcatggaatcggagccatcaagcatacgggtgaggaagtagctgcactgggcgtttcaaaagcgctccttgtcacagaccctgggatttataaagccggtgttgctgatcccgtaatcgaatcacttaaagaagcaggcattgaagtggtactctttaataaagttgagccaaacccgcctgtccgtctggtgaatgaaggatctgagctttacaaaaaagagaactgtaatggtttggtggcagtcggaggcggaagctccatggatacagcaaaagcaatcggagtagaagcgactcacgaaggaagcgtgcttgattatgaagcggcagatgggaaaaaaccgctggaaaaccgcattcctccgctgacgacaattcccactacagctggaaccggatcagaagtaacccaatgggcggttatcacagatgaagaaagagaattcaaattcaacacgggcggtccgctgattgcagcgcacttgacaatcattgatcctgagcttcatgtttcaatgcctccgcatgtaacagctatgacgggaattgatgcgctcgcccatgccattgagtgctatacaatgaaatttgcacagccaatcacggatgcggttgccttaatggcgattgagtatgccgctcattacatcaagagggcatttgctgatggagaggatctggaagcaaggtacggaatggcgcaggctgcgatgcttgccggtctttcttacggaagtgaatcagcgggcgctgctcatgcgatgagccaaacgcttggcggtattatcccagtcgctcacggccaatgtgtagcggcgatgatgggccctgtcatggaatacaactggaagggctatcctgagaagtttgcgcgtattgcgaaagcgttcggtattgatacaagcaagatgacaacagaagaagctgcgaaagcatctgtcaattggatgtatgatctggtcgaagatttagaagtgccgactttagaagagcagggagtatcacctgatatgatcgaacgcttgtctaaagaagcaatgaaagatccgcaaaccttcggaaaccctagagatttaaatgaaaaagcatacaactggatctacaaacgctgctttaaccttacgcctaaaacggtataa

SEQ ID NO: 4 - protein, 402 aa, Bacillus subtilis
MTLNMKVESMQKFHTFEIPTVIKHGIGAIKHTGEEVAALGVSKALLVTDPGIYKAGVADPVIESLKEAGIEVVLFNKVEPNPPVRLVNEGSELYKKENCNGLVAVGGGSSMDTAKAIGVEATHEGSVLDYEAADGKKPLENRIPPLTTIPTTAGTGSEVTQWAVITDEEREFKFNTGGPLIAAHLTIIDPELHVSMPPHVTAMTGIDALAHAIECYTMKFAQPITDAVALMAIEYAAHYIKRAFADGEDLEARYGMAQAAMLAGLSYGSESAGAAHAMSQTLGGIIPVAHGQCVAAMMGPVMEYNWKGYPEKFARIAKAFGIDTSKMTTEEAAKASVNWMYDLVEDLEVPTLEEQGVSPDMIERLSKEAMKDPQTFGNPRDLNEKAYNWIYKRCFNLTPKTV

SEQ ID NO: 5 - DNA, 3254 bp, Artificial
  synthetic DNA
atgaagatttacggaatttatatggaccgcccgctttcacaggaagaaaatgaacggttcatgtctttcatatcacctgaaaaacgggagaaatgccggagattttatcataaagaagatgctcaccgcaccctgctgggagatgtgctcgttcgctcagtcataagcaggcagtatcagttggacaaatccgatatccgctttagcacgcaggaatacgggaagccgtgcatccctgatcttcccgacgctcatttcaacatttctcactccggacgctgggtcatttgcgcgtttgattcacagccgatcggcatagatatcgaaaaaacgaaaccgatcagccttgagatcgccaagcgcttcttttcaaaaacagagtacagcgaccttttagcaaaagacaaggacgagcagacagactatttttatcatctatggtcaatgaaagaaagctttatcaaacaaggaaggcaaaggcttatcgcttccgcttgatttccatcacgcataggcacaacacctaaatgcatgtgaggggtttgctcatcattatgaactgttgcataagcaatattttgcttgccatatcgttcggaaaataatttataactttcctcaaaaaatcgtttttgttctcctggatccggactagtctagagctctacgcgatctccgggcgggcaacgtccgttcattaaaaacaaagccgaaacggttttgtttttaatgaacggacagctttcgtctgatatgataggatggttttgacaatattttcagacggaggatctggacatgaaaatttacggagtatatatggaccgcccgctttctgcaggggaagaggatcggatgatggcggccgtgtccgccgaaaagcgggaaaaatgccggcgcttttaccataaggaggatgctcaccgcaccttgatcggcgacatgctgatccgcaccgctgcggcgaaggcttatggacttgatccggccgggatttcattcggcgtccaggaatacggaaagccgtacatccccgcgcttccggacatgcactttaacatttcccactccgggcgctggatcgtgtgcgccgttgattcaaaaccgatcggcattgatattgaaaaaatgaagcccggcacgattgatatcgccaaacggtttttttcgccgacggaatacagtgatctgcaagcgaaacaccccgatcagcagaccgattatttttaccacctgtggtcgatgaaagaaagctttatcaaacaggccggaaaagggctttccctgccgcttgattcattcagcgtccgcctcaaagacgacggccatgtgtccattgagcttccggacgggcatgaaccttgtttcatccgcacatatgatgcggacgaggagtataagctggccgtttgtgcggcgcatcccgatttttgtgacgggattgagatgaaaacgtatgaagagctgttataagcaatccgtcagcattttgatgcctcgcgtgatatcccctgtcttgacgttggacacgttgagtttgatgatattttctttcggaaaatccgataggtaatggctgtcaatcggctccaccagcacgccttgcgctttcagacgctgcacaactcttgaagcggaaaggcttttctccagcacgagatgggtatggatcgacgtttgctttacagaaaaaccgtcgtactcatcatcggcaatagttacccttattatcaagataagaaagaaaaggatttttcgctacgctcaaatcctttaaaaaaacacaaaagaccacattttttaatgtggtctttattcttcaactaaagcacccattagttcaacaaacgaaaattggataaagtgggatatttttaaaatatatatttatgttacagtaatattgacttttaaaaaaggattgattctaatgaagaaagcagacaagtaagcctcctaaattcactttagataaaaatttaggaggcatatcaaatgaactttaataaaattgatttagacaattggaagagaaaagagatatttaatcattatttgaaccaacaaacgacttttagtataaccacagaaattgatattagtgttttataccgaaacataaaacaagaaggatataaattttaccctgcatttattttcttagtgacaagggtgataaactcaaatacagcttttagaactggttacaatagcgacggagagttaggttattgggataagttagagccactttatacaatttttgatggtgtatctaaaacattctctggtatttggactcctgtaaagaatgacttcaaagagttttatgatttatacctttctgatgtagagaaatataatggttcggggaaattgtttcccaaaacacctatacctgaaaatgctttttctctttctattattccatggacttcatttactgggtttaacttaaatatcaataataatagtaattaccttctacccattattacagcaggaaaattcattaataaaggtaattcaatatatttaccgctatctttacaggtacatcattctgtttgtgatggttatcatgcaggattgtttatgaactctattcaggaattgtcagataggcctaatgactggcttttataatatgagataatgccgactgtactttttacagtcggttttctaatgtcactaacctgccccgttagttgaagaaggtttttatattacagctccagatcctctacgccgccttttcagtgcgcctgcaccaggacggacaagtatccattgagcttccggacagccattccccatgctatatcaaaacgtatgaggtcgatcccggctacaaaatggctgtatgcgccgtacaccctgatttccccgaggatatcacaatggtctcgtacgaagagcttttataaatggctcatcaacagcttgacaccgcgctcaatatcttccgttttcacattggaaatattgatttttaatagattttctttcggataatctgataaataatgacggtctatcgcctcaaggagaaccccttgtttttccagtctatgaatcactcttgaggcgggcagatcctgaggaagcaccagatgggtgtgcatacagggtgcctgcccgctggagaacgtaaagcgtccgcttcccagctgcctgtgagttcgaatggcttgatgtagcctcagcgaccgctctttataagaatctctgattttctccttatgcctgcc

SEQ ID NO: 6 - DNA, 2990 bp, Artificial
  synthetic DNA
gaaacgagtaacccgagacttaatgcactaattgccaaagaagataataatttgcgtttcataacaaaattccccctaaaaaatgataaattaaacaggcctgcccgcttttcacctcctctgaaaggccaaatacaaattttacctacataaaattaccatcaaatattttggaagtaaatggggtgtttttcccgtatttttcaaatttgtagtagttacatcaaaaaaacgcctagtttcccaggcgttttctgctttactttgtttcgaccggtataaatttaaaaatttctccggtctgcaccgattcagcaagccgtttcagccagtcatagtaagctttagagctttccagctgatcatataactgcagtgcttcatttttgatatcctcatcgagatcttccttgcataaaaccttttgtaaatcagcttgagcttcctcgatcgctgttacattcacttgaacctcccgctcccatttaggtggaaagaaatttgtgaaaaatttaaagaaatccttctcagccacaaatgtatgcttgcggatgccccggtgaaatgtttttttcactacatttaagtcttgaagctttttgacgccagtgctcatgcttggtttgctcatttgcaactcctcacgcatttcgtcaagcgtcatctcatccctcatatacatcgtcccatataaaatcccgacactgcgggtaattccgtaaagatccatcgtttcagcaatggagtcaataacaagatcccgagcctgttctatagctgcaaattctggattttcatccatactgaccctcttttcctttagaaaattaaattcgttaagttatttctttatgttctttatcttaacgaaacatgaggaaaagtcaaaaagaaaaatcaaaatgggactttgacagtttaaaaaccatatgttagattaaggttgttaaaaacattaaatttttatttaacaaactttatttacgtcaaggaggcttattcaaaaattatatggagatctgtataataaagaataattattaatctgtagacaaattgtgaaaggatgtacttaaacgctaacggtcagctttattgaacagtaatttaagtatatgtccaatctagggtaagtaaattgagtatcaatataaactttatatgaacataatcaacgaggtgaaatcatgagcaatttgattaacggaaaaataccaaatcaagcgattcaaacattaaaaatcgtaaaagatttatttggaagttcaatagttggagtatatctatttggttcagcagtaaatggtggtttacgcattaacagcgatgtagatgttctagtcgtcgtgaatcatagtttacctcaattaactcgaaaaaaactaacagaaagactaatgactatatcaggaaagattggaaatacggattctgttagaccacttgaagttacggttataaataggagtgaagttgtcccttggcaatatcctccaaaaagagaatttatatacggtgagtggctcaggggtgaatttgagaatggacaaattcaggaaccaagctatgatcctgatttggctattgttttagcacaagcaagaaagaatagtatttctctatttggtcctgattcttcaagtatacttgtctccgtacctttgacagatattcgaagagcaattaaggattctttgccagaactaattgaggggataaaaggtgatgagcgtaatgtaattttaaccctagctcgaatgtggcaaacagtgactactggtgaaattacctcgaaagatgtcgctgcagaatgggctatacctcttttacctaaagagcatgtaactttactggatatagctagaaaaggctatcggggagagtgtgatgataagtgggaaggactatattcaaaggtgaaagcactcgttaagtatatgaaaaattctatagaaacttctctcaattaggctaattttattgcaataacatgacattaaatatgaaggtagaaagcatgcagaaattccacacatttgaaattccgactgtgattaagcatggaatcggagccatcaagcatacgggtgaggaagtagctgcactgggcgtttcaaaagcgctccttgtcacagaccctgggatttataaagccggtgttgctgatcccgtaatcgaatcacttaaagaagcaggcattgaagtggtactctttaataaagttgagccaaacccgcctgtccgtctggtgaatgaaggatctgagctttacaaaaaagagaactgtaatggtttggtggcagtcggaggcggaagctccatggatacagcaaaagcaatcggagtagaagcgactcacgaaggaagcgtgcttgattatgaagcggcagatgggaaaaaaccgctggaaaaccgcattcctccgctgacgacaattcccactacagctggaaccggatcagaagtaacccaatgggcggttatcacagatgaagaaagagaattcaaattcaacacgggcggtccgctgattgcagcgcacttgacaatcattgatcctgagcttcatgtttcaatgcctccgcatgtaacagctatgacgggaattgatgcgctcgcccatgccattgagtgctatacaatgaaatttgcacagccaatcacggatgcggttgccttaatggcgattgagtatgccgctcattacatcaagagggcatttgctgatggagaggatctggaagcaaggtacggaatggcgcaggctgcgatgcttgccggtctttcttacggaagtgaatcagcgggcgctgctcatgcgatgagccaaacgcttggcggtattatcccagtcgctcacggccaatgtgtagcggcgatgatgggccctgtcatggaatacaactggaagggctatcctgagaagtttgcgcgtattgcgaaagcgttcggtattgatacaagcaagatgacaacagaagaagctgcga

SEQ ID NO: 7 - DNA, 2000 bp, Artificial
  synthetic DNA
gaaacgagtaacccgagacttaatgcactaattgccaaagaagataataatttgcgtttcataacaaaattccccctaaaaaatgataaattaaacaggcctgcccgcttttcacctcctctgaaaggccaaatacaaattttacctacataaaattaccatcaaatattttggaagtaaatggggtgtttttcccgtatttttcaaatttgtagtagttacatcaaaaaaacgcctagtttcccaggcgttttctgctttactttgtttcgaccggtataaatttaaaaatttctccggtctgcaccgattcagcaagccgtttcagccagtcatagtaagctttagagctttccagctgatcatataactgcagtgcttcatttttgatatcctcatcgagatcttccttgcataaaaccttttgtaaatcagcttgagcttcctcgatcgctgttacattcacttgaacctcccgctcccatttaggtggaaagaaatttgtgaaaaatttaaagaaatccttctcagccacaaatgtatgcttgcggatgccccggtgaaatgtttttttcactacatttaagtcttgaagctttttgacgccagtgctcatgcttggtttgctcatttgcaactcctcacgcatttcgtcaagcgtcatctcatccctcatatacatcgtcccatataaaatcccgacactgcgggtaattccgtaaagatccatcgtttcagcaatggagtcaataacaagatcccgagcctgttctatagctgcaaattctggattttcatccatactgaccctcttttcctttagaaaattaaattcgttaagttatttctttatgttctttatcttaacgaaacatgaggaaaagtcaaaaagaaaaatcaaaatgggactttgacagtttaaaaaccatatgttagattaaggttgttaaaaacattaaatttttatttaacaaactttatttacgtcaaggaggcttatatgacattaaatatgaaggtagaaagcatgcagaaattccacacatttgaaattccgactgtgattaagcatggaatcggagccatcaagcatacgggtgaggaagtagctgcactgggcgtttcaaaagcgctccttgtcacagaccctgggatttataaagccggtgttgctgatcccgtaatcgaatcacttaaagaagcaggcattgaagtggtactctttaataaagttgagccaaacccgcctgtccgtctggtgaatgaaggatctgagctttacaaaaaagagaactgtaatggtttggtggcagtcggaggcggaagctccatggatacagcaaaagcaatcggagtagaagcgactcacgaaggaagcgtgcttgattatgaagcggcagatgggaaaaaaccgctggaaaaccgcattcctccgctgacgacaattcccactacagctggaaccggatcagaagtaacccaatgggcggttatcacagatgaagaaagagaattcaaattcaacacgggcggtccgctgattgcagcgcacttgacaatcattgatcctgagcttcatgtttcaatgcctccgcatgtaacagctatgacgggaattgatgcgctcgcccatgccattgagtgctatacaatgaaatttgcacagccaatcacggatgcggttgccttaatggcgattgagtatgccgctcattacatcaagagggcatttgctgatggagaggatctggaagcaaggtacggaatggcgcaggctgcgatgcttgccggtctttcttacggaagtgaatcagcgggcgctgctcatgcgatgagccaaacgcttggcggtattatcccagtcgctcacggccaatgtgtagcggcgatgatgggccctgtcatggaatacaactggaagggctatcctgagaagtttgcgcgtattgcgaaagcgttcggtattgatacaagcaagatgacaacagaagaagctgcga

SEQ ID NO: 8 - DNA, 2990 bp, Artificial
  synthetic DNA
gcactggccgcaggaaacacaatcgtcatgaagccgagtgagattacgccgctgacgacaatcaaagtctttaagctgatggaagaagccggtgttccaaaaggtgtcgcaaatcttgttcttggaccgggagccacagtgggcgacgagcttgccgtaaacaaagacgtcgatttgatttcatttacgggcggaattgaaacaggcaaaaaaatcatgcgggcggcaagcggaaacgtcaaaaaaatcgcccttgaacttggcgggaaaaacccaaatattgttttcaaggacgcggatttagaagttgcggttgatcaggccttaaacgctgtatttttccacgccggccaagtatgctctgcaggttcccgcttgcttgttgaggatgccattcatgatcaatttttggcggagctggtcaaacgggcaaaacgcataaaactcggaaacggttttcatgctgagacagaaagcggtccgcttatttcggcggagcacagggcaaaggtagaaaaatatgtagagatcggaatagaggaaggcgcgaagctggagacaggaggcaaacgcccggaagatcctgagcttcaaaacggctttttctatgaacctactattttctcaaactgtaattctgacatgagaatcgttcaggaagaggttttcggtcctgtattgacagtcgaaaccttcagctctgaagaagaggtaatcgagcttgcgaatgataccatctatggcttggctggagcggtatggtcaaaagacattgaaaagtgcgaacgggtagcagcccgcttgagaatgggaaccgtttggatcaacgattttcatccgtactttgcacaagcgccatggggcggatataagcaatccgggttcggacgcgagcttggaaaaataggccttgaagaatacacagaagtcaaacatgtataccgcaatacaaaaccggcagcggttaactggtttaattcataagagggggagattgatgtcaaaaattatatggagatctgtataataaagaataattattaatctgtagacaaattgtgaaaggatgtacttaaacgctaacggtcagctttattgaacagtaatttaagtatatgtccaatctagggtaagtaaattgagtatcaatataaactttatatgaacataatcaacgaggtgaaatcatgagcaatttgattaacggaaaaataccaaatcaagcgattcaaacattaaaaatcgtaaaagatttatttggaagttcaatagttggagtatatctatttggttcagcagtaaatggtggtttacgcattaacagcgatgtagatgttctagtcgtcgtgaatcatagtttacctcaattaactcgaaaaaaactaacagaaagactaatgactatatcaggaaagattggaaatacggattctgttagaccacttgaagttacggttataaataggagtgaagttgtcccttggcaatatcctccaaaaagagaatttatatacggtgagtggctcaggggtgaatttgagaatggacaaattcaggaaccaagctatgatcctgatttggctattgttttagcacaagcaagaaagaatagtatttctctatttggtcctgattcttcaagtatacttgtctccgtacctttgacagatattcgaagagcaattaaggattctttgccagaactaattgaggggataaaaggtgatgagcgtaatgtaattttaaccctagctcgaatgtggcaaacagtgactactggtgaaattacctcgaaagatgtcgctgcagaatgggctatacctcttttacctaaagagcatgtaactttactggatatagctagaaaaggctatcggggagagtgtgatgataagtgggaaggactatattcaaaggtgaaagcactcgttaagtatatgaaaaattctatagaaacttctctcaattaggctaattttattgcaataactcaaaatcccgctcctttacagagcgggattttttgggataatgaagcataggtggaaattttagataagaaggaaggtgccagctgatgtggaagcgtatgactgcaaaagcggaaggcttatatatcgcagatacaaaaagcttcgtaacaaagcaaatggacaagcttgattttgattatggcggcatccccggcgacttgcattttggcctgaccaaaaaagcgggagccagagaaccaatgttttcaagagggactgaaattttcaaccgcagacaaatttcaattgtttcaatagaggaatgcaacgaaatcgctttaaaaatgggagtgccgagaattttgccggaatggctcggggcgaatgtggcagtcagcggtatgccagatcttacttcattaaaagaaggaagccggattatttttccgagcggagcggctctgctgtgtgagggcgaaaatgatccgtgtatccagccgggagaagtcattcagtcttattatccggaccaaccgaagctggcgtcggctttcgtccgccacgcactgggcattagagggattgtctgtattgtggagagacctggtgctgtttacacaggtgatgaaatagaagttcattcctatcagcgaaaagtcaaacgaaaagcagaaagggtctgattaaatcaggccctttctatcttttctttaatttctttcatttggctgaggtgccgtttttcatgatggccgataaaatcgatccactgtctgacagtcagctcttgaaacacaggatgcggaagcactctttcaaaatcttcttctttcagagaggcaatcgcagcagtcagctgctctcttaccacatcaagctcacgtttcatttggctgcctgaaataaaatcatgcgcaggctcaagatgactcggggctttccgtttattatttctgtcctgtgctacttcaagcggtttttcttcaatttctttaatcggagcgtcctttacacgtt

SEQ ID NO: 9 - DNA, 2990 bp, Artificial
  synthetic DNA
gaaacgagtaacccgagacttaatgcactaattgccaaagaagataataatttgcgtttcataacaaaattccccctaaaaaatgataaattaaacaggcctgcccgcttttcacctcctctgaaaggccaaatacaaattttacctacataaaattaccatcaaatattttggaagtaaatggggtgtttttcccgtatttttcaaatttgtagtagttacatcaaaaaaacgcctagtttcccaggcgttttctgctttactttgtttcgaccggtataaatttaaaaatttctccggtctgcaccgattcagcaagccgtttcagccagtcatagtaagctttagagctttccagctgatcatataactgcagtgcttcatttttgatatcctcatcgagatcttccttgcataaaaccttttgtaaatcagcttgagcttcctcgatcgctgttacattcacttgaacctcccgctcccatttaggtggaaagaaatttgtgaaaaatttaaagaaatccttctcagccacaaatgtatgcttgcggatgccccggtgaaatgtttttttcactacatttaagtcttgaagctttttgacgccagtgctcatgcttggtttgctcatttgcaactcctcacgcatttcgtcaagcgtcatctcatccctcatatacatcgtcccatataaaatcccgacactgcgggtaattccgtaaagatccatcgtttcagcaatggagtcaataacaagatcccgagcctgttctatagctgcaaattctggattttcatccatactgaccctcttttcctttagaaaattaaattcgttaagttatttctttatgttctttatcttaacgaaacatgaggaaaagtcaaaaagaaaaatcaaaatgggactttgacagtttaaaaaccatatgttagattaaggttgttaaaaacattaaatttttatttaacaaactttatttacgtcaaggaggcttattcaaaaattatatggagatctgtataataaagaataattattaatctgtagacaaattgtgaaaggatgtacttaaacgctaacggtcagctttattgaacagtaatttaagtatatgtccaatctagggtaagtaaattgagtatcaatataaactttatatgaacataatcaacgaggtgaaatcatgagcaatttgattaacggaaaaataccaaatcaagcgattcaaacattaaaaatcgtaaaagatttatttggaagttcaatagttggagtatatctatttggttcagcagtaaatggtggtttacgcattaacagcgatgtagatgttctagtcgtcgtgaatcatagtttacctcaattaactcgaaaaaaactaacagaaagactaatgactatatcaggaaagattggaaatacggattctgttagaccacttgaagttacggttataaataggagtgaagttgtcccttggcaatatcctccaaaaagagaatttatatacggtgagtggctcaggggtgaatttgagaatggacaaattcaggaaccaagctatgatcctgatttggctattgttttagcacaagcaagaaagaatagtatttctctatttggtcctgattcttcaagtatacttgtctccgtacctttgacagatattcgaagagcaattaaggattctttgccagaactaattgaggggataaaaggtgatgagcgtaatgtaattttaaccctagctcgaatgtggcaaacagtgactactggtgaaattacctcgaaagatgtcgctgcagaatgggctatacctcttttacctaaagagcatgtaactttactggatatagctagaaaaggctatcggggagagtgtgatgataagtgggaaggactatattcaaaggtgaaagcactcgttaagtatatgaaaaattctatagaaacttctctcaattaggctaattttattgcaataactcaaaatcccgctcctttacagagcgggattttttgggataatgaagcataggtggaaattttagataagaaggaaggtgccagctgatgtggaagcgtatgactgcaaaagcggaaggcttatatatcgcagatacaaaaagcttcgtaacaaagcaaatggacaagcttgattttgattatggcggcatccccggcgacttgcattttggcctgaccaaaaaagcgggagccagagaaccaatgttttcaagagggactgaaattttcaaccgcagacaaatttcaattgtttcaatagaggaatgcaacgaaatcgctttaaaaatgggagtgccgagaattttgccggaatggctcggggcgaatgtggcagtcagcggtatgccagatcttacttcattaaaagaaggaagccggattatttttccgagcggagcggctctgctgtgtgagggcgaaaatgatccgtgtatccagccgggagaagtcattcagtcttattatccggaccaaccgaagctggcgtcggctttcgtccgccacgcactgggcattagagggattgtctgtattgtggagagacctggtgctgtttacacaggtgatgaaatagaagttcattcctatcagcgaaaagtcaaacgaaaagcagaaagggtctgattaaatcaggccctttctatcttttctttaatttctttcatttggctgaggtgccgtttttcatgatggccgataaaatcgatccactgtctgacagtcagctcttgaaacacaggatgcggaagcactctttcaaaatcttcttctttcagagaggcaatcgcagcagtcagctgctctcttaccacatcaagctcacgtttcatttggctgcctgaaataaaatcatgcgcaggctcaagatgactcggggctttccgtttattatttctgtcctgtgctacttcaagcggtttttcttcaatttctttaatcggagcgtcctttacacgtt